European Patent Application EP 4 349 991 A1, published April 10, 2024. Title: Strain for producing high concentration L-glutamic acid and method for producing L-glutamic acid using the same. Applicant: CJ CheilJedang Corporation. The sequence listing filed with the application follows.

SEQUENCE LISTING (32 sequences)

SEQ ID NO: 1 - protein, 196 aa, Unknown
  VKOR
MSTEIHNAPPKAPTWLGWVLMIGGIIGLILSVIIMAEKLAILEDPGHITSCDFNAVLACGDVMRSGQANAFGIPNPLIGIAGFAAVAIIGAGILAGGRFRGWFWFGAQAGLTFAMMFCHWLAYQSMSVIRALCPYCMGVWTVSIIMFVLVTAWNVKTFSGSDSTFVNALYKYKWVIAIVWLLLIAAAAVWSFRYMF

SEQ ID NO: 2 - DNA, 591 bp, Unknown
  VKOR
gtgtctaccgaaatccacaacgccccacccaaggccccaacttggcttggctgggtgctcatgatcggcggaataatcggcctcattttgtcggtgatcatcatggccgaaaaacttgccatcctcgaggatcccggtcacatcaccagctgcgatttcaatgcagtcctagcttgtggcgatgtcatgcgttccggccaagctaacgcgttcggcatcccgaatccgctcatcggcatcgccggtttcgccgctgtcgccatcatcggcgccggcatcctcgcgggcggcaggttccgcggttggttctggttcggcgcccaggccggactcacttttgccatgatgttctgccactggctcgcctaccaatccatgtccgtcatccgcgcgctctgcccttactgcatgggcgtgtggaccgtatcgatcatcatgttcgtgctggtcactgcatggaatgtgaaaactttcagcggctccgacagcacgttcgtcaacgcactgtacaaatacaagtgggtcatcgcgatcgtctggctgctgctcatcgcagccgcagctgtgtggtcattccgctacatgttctag

SEQ ID NO: 3 - DNA, 38 bp, Artificial Sequence
  odhA_up_F
tgaattcgagctcggtacccttgaacggaattgggtgg

SEQ ID NO: 4 - DNA, 38 bp, Artificial Sequence
  odhA_up_R
cccaggtggcatcggtaccttcacccagcgccacgcag

SEQ ID NO: 5 - DNA, 39 bp, Artificial Sequence
  odhA_down_F
cgctgggtgaaggtaccgatgccacctgggttggtcaag

SEQ ID NO: 6 - DNA, 38 bp, Artificial Sequence
  odhA_down_R
gtcgactctagaggatccccggacaaggaatggagaga

SEQ ID NO: 7 - DNA, 18 bp, Artificial Sequence
  odhA_del_F
cttaccgttgttgccctt

SEQ ID NO: 8 - DNA, 19 bp, Artificial Sequence
  odhA_del_R
ctccttcacccacatcatt

SEQ ID NO: 9 - DNA, 25 bp, Artificial Sequence
  primer 1
acctacaacaaagctctcatcaacc

SEQ ID NO: 10 - DNA, 24 bp, Artificial Sequence
  primer 2
ctaccctgtggaacacctacatct

SEQ ID NO: 11 - DNA, 39 bp, Artificial Sequence
  BBD29_04485_up_F
aattcgagctcggtacccgtgagtccaaccaggtcgaag

SEQ ID NO: 12 - DNA, 39 bp, Artificial Sequence
  BBD29_04485_up_R
ctgaaagccttaaatgctggcttgatttcttgtgctgtg

SEQ ID NO: 13 - DNA, 37 bp, Artificial Sequence
  BBD29_04485_down_F
acaagaaatcaagccagcatttaaggctttcaggccg

SEQ ID NO: 14 - DNA, 40 bp, Artificial Sequence
  BBD29_04485_down_R
cgactctagaggatccccgtatcgacaagggtgagtgatg

SEQ ID NO: 15 - DNA, 38 bp, Artificial Sequence
  BBD29_04485_up_F_2
ttcgagctcggtacccgttgatgatcagggaaggctgt

SEQ ID NO: 16 - DNA, 38 bp, Artificial Sequence
  BBD29_04485_up_R_2
tggatttcggtagacaaggggagacctccgggtgggaa

SEQ ID NO: 17 - DNA, 38 bp, Artificial Sequence
  BBD29_04485_down_F_2
acccggaggtctccccttgtctaccgaaatccacaacg

SEQ ID NO: 18 - DNA, 38 bp, Artificial Sequence
  BBD29_04485_down_R_2
actctagaggatcccctcggtcaggtgtgtgtaaatag

SEQ ID NO: 19 - DNA, 38 bp, Artificial Sequence
  BBD29_04485_up_R_3
tggatttcggtagacagggggagacctccgggtgggaa

SEQ ID NO: 20 - DNA, 38 bp, Artificial Sequence
  BBD29_04485_down_F_3
acccggaggtctccccctgtctaccgaaatccacaacg

SEQ ID NO: 21 - DNA, 38 bp, Artificial Sequence
  BBD29_04485_up_F_4
ttcgagctcggtaccccagcatcttcttcttcgccgaa

SEQ ID NO: 22 - DNA, 40 bp, Artificial Sequence
  BBD29_04485_up_R_4
gtagacacggggagaactttcgaggggaaaacgtttgttg

SEQ ID NO: 23 - DNA, 40 bp, Artificial Sequence
  BBD29_04485_down_F_4
aacaaacgttttcccctcgaaagttctccccgtgtctacc

SEQ ID NO: 24 - DNA, 38 bp, Artificial Sequence
  BBD29_04485_down_R_4
actctagaggatcccccttttctgagctggaggaacaa

SEQ ID NO: 25 - DNA, 40 bp, Artificial Sequence
  BBD29_04485_up_R_5
gtagacacggggagagcctcgagtgggaaaacgtttgttg

SEQ ID NO: 26 - DNA, 40 bp, Artificial Sequence
  BBD29_04485_down_F_5
aacaaacgttttcccactcgaggctctccccgtgtctacc

SEQ ID NO: 27 - DNA, 40 bp, Artificial Sequence
  BBD29_04485_up_R_6
gtagacacggggagagtccagggcgggaaaacgtttgttg

SEQ ID NO: 28 - DNA, 40 bp, Artificial Sequence
  BBD29_04485_down_F_6
aacaaacgttttcccgccctggactctccccgtgtctacc

SEQ ID NO: 29 - DNA, 19 bp, Artificial Sequence
  BBD29_04485_del_F
ataatccaccaaaactgcc

SEQ ID NO: 30 - DNA, 19 bp, Artificial Sequence
  BBD29_04485_del_R
aggtgtgtgtaaataggga

SEQ ID NO: 31 - DNA, 18 bp, Artificial Sequence
  BBD29_04485_seq_F
gtggttgtcttcgatagt

SEQ ID NO: 32 - protein, 1205 aa, Unknown
  OdhA
MFQQFQKDPKSVDKEWRELFEAQGGPNATPATTEAQPSAPKESAKPAPKAAPAAKAAPRVETKPAAKTAPKAKESSVPQQPKLPEPGQTPIRGIFKSIAKNMDISLEIPTATSVRDMPARLMFENRAMVNDQLKRTRGGKISFTHIIGYAMVKAVMAHPDMNNSYDVIDGKPTLIVPEHINLGLAIDLPQKDGSRALVVAAIKETEKMNFSEFLAAYEDIVTRSRKGKLTMDDYQGVTVSLTNPGGIGTRHSVPRLTKGQGTIIGVGSMDYPAEFQGASEDRLAELGVGKLVTITSTYDHRVIQGAVSGEFLRTMSRLLTDDSFWDEIFDAMNVPYTPMRWAQDVPNTGVDKNTRVMQLIEAYRSRGHLIADTNPLSWVQPGMPVPDHRDLDIETHSLTIWDLDRTFSVGGFGGKETMTLREVLSRLRAAYTLKVGSEYTHILDRDERTWLQDRLEAGMPKPTQAEQKYILQKLNAAEAFENFLQTKYVGQKRFSLEGAEALIPLMDSAIDTAAGQGLDEVVIGMPHRGRLNVLFNIVGKPLASIFNEFEGQMEQGQIGGSGDVKYHLGSEGQHLQMFGDGEIKVSLTANPSHLEAVNPVMEGIVRAKQDYLDKGVDGKTVVPLLLHGDAAFAGLGIVPETINLAKLRGYDVGGTIHIVVNNQIGFTTTPDSSRSMHYATDYAKAFGCPVFHVNGDDPEAVVWVGQLATEYRRRFGKDVFIDLVCYRLRGHNEADDPSMTQPKMYELITGRETVRAQYTEDLLGRGDLSNEDAEAVVRDFHDQMESVFNEVKEGGKKQAEAQTGITGSQKLPHGLETNISREELLELGQAFANTPEGFNYHPRVAPVAKKRVSSVTEGGIDWAWGELLAFGSLANSGRLVRLAGEDSRRGTFTQRHAVAIDPATAEEFNPLHELAQSKGNNGKFLVYNSALTEYAGMGFEYGYSVGNEDSVVAWEAQFGDFANGAQTIIDEYVSSGEAKWGQTSKLILLLPHGYEGQGPDHSSARIERFLQLCAEGSMTVAQPSTPANHFHLLRRHALSDLKRPLVIFTPKSMLRNKAAASAPEDFTEVTKFQSVIDDPNVADAAKVKKVMLVSGKLYYELAKRKEKDGRDDIAIVRIEMLHPIPFNRISEALAGYPNAEEVLFVQDEPANQGPWPFYQEHLPELIPNMPKMRRVSRRAQSSTATGVAKVHQLEEKQLIDEAFEA